European Patent Application EP 4 328 237 A1, published February 28, 2024. Title: Modified polypeptide having lysozyme activity. Applicant: CJ CheilJedang Corporation. The sequence listing filed with the application follows.

SEQUENCE LISTING (14 sequences)

SEQ ID NO: 1 - protein, 233 aa, Artificial Sequence
  Ps_Lys_nt
MKFSSLVVASILGFAAATPASLEKRATVQGFDISGYQPTVDFAGAYASGARFVIIKATEGTSYKSPVFSSQYTGATKAGFIRGAYHFAHPGSSSGAAQANYFLANGGGWSKDGITLPGMLDIEYNPSGATCFGISQSAMVAWIKDFVNTYHTKTGVYPLIYTTTDWWTQCTGNNASFGSTCPLVLARYSTSPGTMPAGWAFQTIWQNNDAYKYGGDSDIFNGSLDQLKKIALG

SEQ ID NO: 2 - DNA, 699 bp, Artificial Sequence
  Ps_Lys_nt
atgaagttctcgagtcttgtcgtcgcgtccattcttggattcgccgccgctacacctgcttcacttgagaagcgggccacggtgcagggtttcgacatatcgggttaccaaccgacggtggacttcgcgggtgcatacgcttcgggggcgagattcgtcatcataaaagcaaccgaaggcacgtcttataaatcgcctgtattctcctcccaatacacaggtgcaactaaagccggatttatcagaggcgcgtatcactttgcccaccccggaagttcgagtggagcagcccaggccaactactttctggcaaacggtggaggatggagcaaagacggcataacgttgccggggatgctggatatcgagtacaatccgtcgggggccacctgtttcggtatatcacagtcggcaatggttgcatggattaaggacttcgtgaacacttaccatacaaaaaccggagtttacccgttgatatatactaccaccgactggtggactcagtgcacggggaataacgcatcgttcgggtcgacatgcccgttagtcttggcacggtattctacatccccaggtacgatgccagcagggtgggcgtttcaaacaatatggcagaataatgatgcttacaagtatggcggtgattcagacattttcaacggctctctggatcagcttaaaaagatcgcgcttggt

SEQ ID NO: 3 - protein, 216 aa, Artificial Sequence
  Ps_Lys_mature
TPASLEKRATVQGFDISGYQPTVDFAGAYASGARFVIIKATEGTSYKSPVFSSQYTGATKAGFIRGAYHFAHPGSSSGAAQANYFLANGGGWSKDGITLPGMLDIEYNPSGATCFGISQSAMVAWIKDFVNTYHTKTGVYPLIYTTTDWWTQCTGNNASFGSTCPLVLARYSTSPGTMPAGWAFQTIWQNNDAYKYGGDSDIFNGSLDQLKKIALG

SEQ ID NO: 4 - DNA, 24 bp, Artificial Sequence
  PICZ_F
tgagtttgtagccttagacatgac

SEQ ID NO: 5 - DNA, 21 bp, Artificial Sequence
  PICZ_R
agcttcagcctctcttttctc

SEQ ID NO: 6 - DNA, 37 bp, Artificial Sequence
  Ps_Lys_F1
aagagaggctgaagctacacctgcttcacttgagaag

SEQ ID NO: 7 - DNA, 37 bp, Artificial Sequence
  Ps_Lys_R1
taaggctacaaactcaaccaagcgcgatctttttaag

SEQ ID NO: 8 - DNA, 22 bp, Artificial Sequence
  S118P_F
gtttcggtataccacagtcggc

SEQ ID NO: 9 - DNA, 22 bp, Artificial Sequence
  S118P_R
gccgactgtggtataccgaaac

SEQ ID NO: 10 - DNA, 22 bp, Artificial Sequence
  Q185L_F
gtgggcgtttttgacaatatgg

SEQ ID NO: 11 - DNA, 22 bp, Artificial Sequence
  Q185L_R
ccatattgtcaaaaacgcccac

SEQ ID NO: 12 - protein, 216 aa, Artificial Sequence
  Ps_Lys_Mature S118P
TPASLEKRATVQGFDISGYQPTVDFAGAYASGARFVIIKATEGTSYKSPVFSSQYTGATKAGFIRGAYHFAHPGSSSGAAQANYFLANGGGWSKDGITLPGMLDIEYNPSGATCFGIPQSAMVAWIKDFVNTYHTKTGVYPLIYTTTDWWTQCTGNNASFGSTCPLVLARYSTSPGTMPAGWAFQTIWQNNDAYKYGGDSDIFNGSLDQLKKIALG

SEQ ID NO: 13 - protein, 216 aa, Artificial Sequence
  Ps_Lys_Mature Q185L
TPASLEKRATVQGFDISGYQPTVDFAGAYASGARFVIIKATEGTSYKSPVFSSQYTGATKAGFIRGAYHFAHPGSSSGAAQANYFLANGGGWSKDGITLPGMLDIEYNPSGATCFGISQSAMVAWIKDFVNTYHTKTGVYPLIYTTTDWWTQCTGNNASFGSTCPLVLARYSTSPGTMPAGWAFLTIWQNNDAYKYGGDSDIFNGSLDQLKKIALG

SEQ ID NO: 14 - protein, 216 aa, Artificial Sequence
  Ps_Lys_Mature S118P+Q185L
TPASLEKRATVQGFDISGYQPTVDFAGAYASGARFVIIKATEGTSYKSPVFSSQYTGATKAGFIRGAYHFAHPGSSSGAAQANYFLANGGGWSKDGITLPGMLDIEYNPSGATCFGIPQSAMVAWIKDFVNTYHTKTGVYPLIYTTTDWWTQCTGNNASFGSTCPLVLARYSTSPGTMPAGWAFLTIWQNNDAYKYGGDSDIFNGSLDQLKKIALG